European Patent Specification EP 4 175 463 B1, published May 28, 2025. Title: BREMIA LACTUCAE RESISTANCE SG01. Applicant: Syngenta Crop Protection AG de Lange, Michel  Norbert Alexander Lokossou, Anoma Akuvi. The sequence listing filed with the application follows.

SEQUENCE LISTING (20 sequences)

SEQ ID NO: 1 - DNA, 155 bp, Lactuca sativa
  misc_feature (2)..(2): n is A, T, C, or G
  misc_feature (51)..(51): n is A, T, C, or G
  misc_feature (90)..(90): n is A, T, C, or G
  misc_feature (101)..(101): n is A, T, C, or G
  misc_feature (112)..(112): r is A or G
tntaaagattagatacagggcagggaggaatgcctttgagataaatgaggngatcgacagtgtcatgagacgatacaaagagatcaaccnggcagatcatncaattcctccrggaagggttgattccatgaagccatccacatcaacaccatcag

SEQ ID NO: 2 - DNA, 22 bp, Synthetic
agatacagggcagggaggaatg

SEQ ID NO: 3 - DNA, 15 bp, Synthetic
acccttcccggagga

SEQ ID NO: 4 - DNA, 16 bp, Synthetic
caacccttcctggagg

SEQ ID NO: 5 - DNA, 23 bp, Synthetic
tgatgtggatggcttcatggaat

SEQ ID NO: 6 - DNA, 157 bp, Lactuca sativa
  misc_feature (101)..(101): n is A, T, C, or G
  misc_feature (104)..(104): n is A, T, C, or G
  misc_feature (112)..(112): r is A or G
ggtacacgctcgcagtgaaagccttggagataactcaggagatcgatcatgccatgaaacaactctctcagatagaatggactgatgattcagttcctttnggnagaaatgrttccacaaaggcatccacctctacaccatcaagtgattacaatga

SEQ ID NO: 7 - DNA, 21 bp, Synthetic
cgcagtgaaagccttggagat

SEQ ID NO: 8 - DNA, 19 bp, Synthetic
tgcctttgtggaatcattt

SEQ ID NO: 9 - DNA, 18 bp, Synthetic
cctttgtggaaccatttc

SEQ ID NO: 10 - DNA, 22 bp, Synthetic
cacttgatggtgtagaggtgga

SEQ ID NO: 11 - DNA, 138 bp, Lactuca sativa
  misc_feature (41)..(41): n is A, T, C, or G
  misc_feature (62)..(62): n is A, T, C, or G
  misc_feature (99)..(99): r is A or G
gcacttgcaagcatgagacagctcgaagagttaactataanatattgcaaggccttgaaagngattgtgaagaaggaagaagacaatgcatcatcatcntcatcgaaggaggttgtggtcttgcctcatctaaagtcc

SEQ ID NO: 12 - DNA, 21 bp, Synthetic
gcatgagacagctcgaagagt

SEQ ID NO: 13 - DNA, 18 bp, Synthetic
ccttcgatgacgatgatg

SEQ ID NO: 14 - DNA, 19 bp, Synthetic
tccttcgatgatgatgatg

SEQ ID NO: 15 - DNA, 18 bp, Synthetic
tgaggcaagaccacaacc

SEQ ID NO: 16 - DNA, 80 bp, Lactuca sativa
  misc_feature (6)..(6): n is A, T, C, or G
  misc_feature (6)..(6): m is A or C
  misc_feature (41)..(41): n is a, c, g, or t
agacgntttaacgacctggcccaacattccatgaaccaccngactggttttgggcaatttagtcgggtacctgcctttgc

SEQ ID NO: 17 - DNA, 20 bp, Synthetic
acgacctggcccaacattcc

SEQ ID NO: 18 - DNA, 15 bp, Synthetic
tgaaccacccgactg

SEQ ID NO: 19 - DNA, 16 bp, Synthetic
tgaaccaccagactgg

SEQ ID NO: 20 - DNA, 22 bp, Synthetic
gtacccgactaaattgcccaaa